European Patent Application EP 4 596 678 A1, published August 6, 2025. Title: 工程化的间充质干细胞及其用途. Applicant: 清华大学. The sequence listing filed with the application follows.

SEQUENCE LISTING (11 sequences)

SEQ ID NO: 1 - DNA, 822 bp, Mus musculus
  source 1..822: mol_type = genomic DNA
atggcggcgagaagagccctgattgtactggcccattcagagaagacatcattcaactacgccatgaaggaggctgctgtagaggctctgaagaagagaggatgggaggtactcgaatctgacctctatgctatgaacttcaaccccatcatttccagaaatgacatcacaggtgagctgaaggactcgaagaactttcagtatccttccgagtcatctctagcatataaggaaggacgcctgagcccagatattgtggccgaacacaagaagctggaagctgcagacctggtgatatttcagttcccattgcagtggtttggggtgccagccattctgaaaggctggtttgagagagtgctcgtagcaggatttgcctacacatatgctgccatgtacgacaacggtcctttccagaataagaagaccttgctttctatcaccactgggggtagcggctccatgtactctcttcagggtgtccacggggacatgaacgtcattctctggccgattcagagtggcatcctgcgtttctgtggcttccaggtcttagaacctcaactggtttacagcattggccacactccaccagatgcccgcatgcagatcctggaaggatggaagaaacgtctggaaaccgtctgggaggagaccccactctattttgctccaagcagcctgtttgacctaaactttcaggcaggattcttaatgaaaaaggaagttcaagaggagcagaagaagaacaagtttggcctctctgtgggccatcacctgggcaagtccattccagctgacaaccagatcaaagctagaaaa

SEQ ID NO: 2 - DNA, 68 bp, synthetic construct
  source 1..68: mol_type = other DNA
agggccggacgtggggccccagagcgacgctgagtgcgtgcgggactcggagtacgtgacggagcccc

SEQ ID NO: 3 - DNA, 197 bp, synthetic construct
  source 1..197: mol_type = other DNA
tgcatctcaattagtcagcaaccatagtcccgcccctaactccgcccatcccgcccctaactccgcccagttccgcccattctccgccccatggctgactaattttttttatttatgcagaggccgaggccgcctcggcctctgagctattccagaagtagtgaggaggcttttttggaggcctaggcttttgcaaa

SEQ ID NO: 4 - DNA, 1158 bp, synthetic construct
  source 1..1158: mol_type = other DNA
atggagacagacacactcctgctatgggtactgctgctctgggttccaggttccactggttcgcgagcccctacaagcagcagcaccaagaagacccagctgcagctggaacacctgctgctggatctgcagatgatcctgaacggcatcaacaactacaagaaccccaagctgacccggatgctgaccgccaagttctacatgcccaagaaggccaccgagctgaagcacctccagtgtctggaggaggagctgaagcctctggaggaagtgctgaacctggcccagagcaagaacttccacttcgaccccagggacgtggtgtccaacatcaacgtgttcgtgctggaactgaagggcagcgagaccaccttcatgtgcgagtacgccgacgagaccgctaccatcgtggagttcctgaaccgctggatcaccttttgccagagcatcatcagcacactgaccttcgaagacaaaactcacacatgcccaccgtgcccagcacctgaactcctggggggaccgtcagtcttcctcttccccccaaaacccaaggacaccctcatgatctcccggacccctgaggtcacatgcgtggtggtggacgtgagccacgaagaccctgaggtcaagttcaactggtacgtggacggcgtggaggtgcataatgccaagacaaagccgcgggaggagcagtacaacagcacgtaccgtgtggtcagcgtcctcaccgtcctgcaccaggactggctgaatggcaaggagtacaagtgcaaggtctccaacaaagccctcccagcccccatcgagaaaaccatctccaaagccaaagggcagccccgagaaccacaggtgtacaccctgcccccatcccgggatgagctgaccaagaaccaggtcagcctgacctgcctggtcaaaggcttctatcccagcgacatcgccgtggagtgggagagcaatgggcagccggagaacaactacaagaccacgcctcccgtgctggactccgacggctccttcttcctctacagcaagctcaccgtggacaagagcaggtggcagcaggggaacgtcttctcatgctccgtgatgcatgaggctctgcacaaccactacacgcagaagagcctctccctgtctccgggtaaataatag

SEQ ID NO: 5 - DNA, 1244 bp, synthetic construct
  source 1..1244: mol_type = other DNA
atggagacagacacactcctgctatgggtactgctgctctgggttccaggttccactggttcgcgacgtacggtgcctatcagacagctccactaccgcctgcgcgacgagcagcagaagtccctggtgctgtctgacccatacgagctcaaggctctccacctcaacggccagaacattaaccagcaggtgattttctctatgtccttcgtgcagggcgagccatctaacgacaagatcccagtggccctcgggctcaagggaaagaacctgtacctctcttgcgtgatgaaggacggaacccctacactgcagctggagagcgtggacccaaagcagtaccctaagaagaagatggagaagcggttcgtgttcaacaagattgaggtgaagtctaaggtggagttcgagagcgctgagttcccaaactggtacattagcacatctcaggccgagcacaagccagtgttcctcggaaacaactccgggcaggacattattgacttcaccatggagtccgtgtcctccggatcaggtgaacctaagagcagcgacaagacccacacttgccccccttgtcccgctccggaaactcctgggcggaccgtcagtcttcctcttccccccaaaacccaaggacaccctcatgatctcccggacccctgaggtcacatgcgtggtggtggacgtgagccacgaagaccctgaggtcaagttcaactggtacgtggacggcgtggaggtgcataatgccaagacaaagccgcgggaggagcagtacaacagcacgtaccgtgtggtcagcgtcctcaccgtcctgcaccaggactggctgaatggcaaggagtacaagtgcaaggtctccaacaaagccctcccagcccccatcgagaaaaccatctccaaagccaaagggcagccccgagaaccacaggtgtacaccctgcccccatcccgggatgagctgaccaagaaccaggtcagcctgacctgcctggtcaaaggcttctatcccagcgacatcgccgtggagtgggagagcaatgggcagccggagaacaactacaagaccacgcctcccgtgttggactccgacggctccttcttcctctacagcaagctcaccgtggacaagagcaggtggcagcaggggaacgtcttctcatgctccgtgatgcatgaggctctgcacaaccactacacgcagaagagcctctccctgtctccgggtaaataatgaattc

SEQ ID NO: 6 - DNA, 33 bp, synthetic construct
  source 1..33: mol_type = other DNA
gccctacgtgctgtctcacacagcctgtctgac

SEQ ID NO: 7 - DNA, 35 bp, synthetic construct
  source 1..35: mol_type = other DNA
ccacagtgcatacgtgggctccaacaggtcctctt

SEQ ID NO: 8 - DNA, 24 bp, synthetic construct
  source 1..24: mol_type = other DNA
gacgtgacaaacgaagccgacgtc

SEQ ID NO: 9 - DNA, 24 bp, synthetic construct
  source 1..24: mol_type = other DNA
acacgtgggttcccgcacgtccgc

SEQ ID NO: 10 - DNA, 19 bp, synthetic construct
  source 1..19: mol_type = other DNA
gacgtgactcggaccacat

SEQ ID NO: 11 - DNA, 31 bp, synthetic construct
  source 1..31: mol_type = other DNA
gcccacacgctcggtgcgtgcccagttgaac